European Patent Specification EP 3 940 077 B1, published January 1, 2025. Title: Simultaneous surface display vector of dual antigen using. Applicant: SEWON. The sequence listing filed with the application follows.

SEQUENCE LISTING (34 sequences)

SEQ ID NO: 1 - DNA, 406 bp, Lactobacillus casei
ccatgcaatacccacttattgcgatttgcttttctattagttagcattttaaattgtgaaacgtgccacttataaacaaatttccgtcttctttttatgagagtaatctcatttaatcttgactaaatatccgattgcggtcacacaactaccagtttcaaacaaatttcaatttgatggtcattttttattttgtcggcaaaaagtgagcaaatcagtagcattttccctgattacggggtacattcaaagtgactttgcgtacacacagacatatgtatgacgggtgttataaaaagccgtcacgctgctcgagtagctctcatcattttctcgcccttttctcccgcaacatatgataaaatacaacggttgtgaattgtttatttcctaggaggatatctac

SEQ ID NO: 2 - DNA, 607 bp, Lactobacillus casei
aattcagcaagccgcaatacaatgtttctgttttgaagcttgaagttccagttgatcaaaagtttgttgaaggctacaccgatgacggcgttacccctgtttacagcaaggaagaagccgctaagtattacaaggaacagtcagatgcaacggatctcccattcatcttcctgtccgctggtgtcaccaacgaattgttccttgaagaactcaagtttgctaagcaagcaggttcagcctttaatggtgttctctgtggccgtgcaacttggaagccgggtgttaagccatatgctgctgaaggcgaagctgctggtaagaagtggctgcagaccgaaggcaaggctaacattgatcgtttgaacaaggtgcttgcagaaactgcaaccccttggactgacaaagttgaaggttaatctttaaccatagttgcaagaaaggaccgattatgatgatcggttctttttttatgactgcggacatgtttttgtgaccactgcaaacatcaaaatgaagttcgaaaaacttgctaacaatcattacaggtcagtgatccagtggtagactggtattgaatgcgttttcgtctattaggaggtaattcaac

SEQ ID NO: 3 - DNA, 31 bp, Artificial Sequence
  Forward primer
tggtggatccgtgagcaagggcgaggagctg

SEQ ID NO: 4 - DNA, 47 bp, Artificial Sequence
  Reverse primer
tgactctagaactagtgtcgacggtaccttacttgtacagctcgtcc

SEQ ID NO: 5 - DNA, 30 bp, Artificial Sequence
  Forward primer
tacggcatgcttgaattggtttcttacgat

SEQ ID NO: 6 - DNA, 30 bp, Artificial Sequence
  Reverse primer
tacgctcgaggttgaattacctcctaatag

SEQ ID NO: 7 - DNA, 29 bp, Artificial Sequence
  Forward primer
gcgcgaattcttgaattggtttcttacga

SEQ ID NO: 8 - DNA, 28 bp, Artificial Sequence
  Reverse primer
gcgctgcgcattacttgtacagctcgtc

SEQ ID NO: 9 - DNA, 31 bp, Artificial Sequence; identical to SEQ ID NO: 3
  PCR primer

SEQ ID NO: 10 - DNA, 47 bp, Artificial Sequence; identical to SEQ ID NO: 4
  PCR primer

SEQ ID NO: 11 - DNA, 34 bp, Artificial Sequence
  PCR primer
tcgagcatgcaatacccacttattgcgatttgct

SEQ ID NO: 12 - DNA, 74 bp, Artificial Sequence
  PCR primer
tacgggatccaccagaaccaccagaaccaccagaaccaccagaaccacctgagagtacgtcgtcagaatacgtt

SEQ ID NO: 13 - DNA, 34 bp, Artificial Sequence; identical to SEQ ID NO: 11
  PCR primer

SEQ ID NO: 14 - DNA, 74 bp, Artificial Sequence
  PCR primer
tacgggatccaccagaaccaccagaaccaccagaaccaccagaaccacctcccatcataatatcgcctacaaat

SEQ ID NO: 15 - DNA, 34 bp, Artificial Sequence; identical to SEQ ID NO: 11
  PCR primer

SEQ ID NO: 16 - DNA, 74 bp, Artificial Sequence
  PCR primer
tacgggatccaccagaaccaccagaaccaccagaaccaccagaaccacctttttgctccgttactttttcaaca

SEQ ID NO: 17 - DNA, 34 bp, Artificial Sequence; identical to SEQ ID NO: 11
  PCR primer

SEQ ID NO: 18 - DNA, 74 bp, Artificial Sequence
  PCR primer
tacgggatccaccagaaccaccagaaccaccagaaccaccagaaccacctgctacataatccgaggctctaaag

SEQ ID NO: 19 - DNA, 34 bp, Artificial Sequence; identical to SEQ ID NO: 11
  PCR primer

SEQ ID NO: 20 - DNA, 74 bp, Artificial Sequence
  PCR primer
tacgggatccaccagaaccaccagaaccaccagaaccaccagaaccaccgactttctggtacgaaattttcttt

SEQ ID NO: 21 - DNA, 180 bp, Artificial Sequence
  PgsA1
atgaaaaaagaactgagctttcatgaaaagctgctaaagctgacaaaacagcaaaaaaagaaaaccaataagcacgtatttattgccattccgatcgtttttgtccttatgttcgctttcatgtgggcgggaaaagcggaaacgccgaaggtcaaaacgtattctgacgacgtactctca

SEQ ID NO: 22 - DNA, 210 bp, Artificial Sequence
  PgsA2
atgaaaaaagaactgagctttcatgaaaagctgctaaagctgacaaaacagcaaaaaaagaaaaccaataagcacgtatttattgccattccgatcgtttttgtccttatgttcgctttcatgtgggcgggaaaagcggaaacgccgaaggtcaaaacgtattctgacgacgtactctcagcctcatttgtaggcgatattatgatggga

SEQ ID NO: 23 - DNA, 240 bp, Artificial Sequence
  PgsA3
atgaaaaaagaactgagctttcatgaaaagctgctaaagctgacaaaacagcaaaaaaagaaaaccaataagcacgtatttattgccattccgatcgtttttgtccttatgttcgctttcatgtgggcgggaaaagcggaaacgccgaaggtcaaaacgtattctgacgacgtactctcagcctcatttgtaggcgatattatgatgggacgctatgttgaaaaagtaacggagcaaaaa

SEQ ID NO: 24 - DNA, 300 bp, Artificial Sequence
  PgsA4
atgaaaaaagaactgagctttcatgaaaagctgctaaagctgacaaaacagcaaaaaaagaaaaccaataagcacgtatttattgccattccgatcgtttttgtccttatgttcgctttcatgtgggcgggaaaagcggaaacgccgaaggtcaaaacgtattctgacgacgtactctcagcctcatttgtaggcgatattatgatgggacgctatgttgaaaaagtaacggagcaaaaaggggcagacagtatttttcaatatgttgaaccgatctttagagcctcggattatgtagca

SEQ ID NO: 25 - DNA, 564 bp, Artificial Sequence
  PgsA5
atgaaaaaagaactgagctttcatgaaaagctgctaaagctgacaaaacagcaaaaaaagaaaaccaataagcacgtatttattgccattccgatcgtttttgtccttatgttcgctttcatgtgggcgggaaaagcggaaacgccgaaggtcaaaacgtattctgacgacgtactctcagcctcatttgtaggcgatattatgatgggacgctatgttgaaaaagtaacggagcaaaaaggggcagacagtatttttcaatatgttgaaccgatctttagagcctcggattatgtagcaggaaactttgaaaacccggtaacctatcaaaagaattataaacaagcagataaagagattcatctgcagacgaataaggaatcagtgaaagtcttgaaggatatgaatttcacggttctcaacagcgccaacaaccacgcaatggattacggcgttcagggcatgaaagatacgcttggagaatttgcgaagcaaaaccttgatatcgttggagcgggatacagcttaagtgatgcgaaaaagaaaatttcgtaccagaaagtc

SEQ ID NO: 26 - DNA, 38 bp, Artificial Sequence
  PCR primer
cgctggatatctacatgcacgtatttattgccattccg

SEQ ID NO: 27 - DNA, 74 bp, Artificial Sequence; identical to SEQ ID NO: 12
  PCR primer

SEQ ID NO: 28 - DNA, 38 bp, Artificial Sequence; identical to SEQ ID NO: 26
  PCR primer

SEQ ID NO: 29 - DNA, 74 bp, Artificial Sequence; identical to SEQ ID NO: 14
  PCR primer

SEQ ID NO: 30 - DNA, 38 bp, Artificial Sequence; identical to SEQ ID NO: 26
  PCR primer

SEQ ID NO: 31 - DNA, 74 bp, Artificial Sequence; identical to SEQ ID NO: 18
  PCR primer

SEQ ID NO: 32 - DNA, 108 bp, Artificial Sequence
  PgsA6
cacgtatttattgccattccgatcgtttttgtccttatgttcgctttcatgtgggcgggaaaagcggaaacgccgaaggtcaaaacgtattctgacgacgtactctca

SEQ ID NO: 33 - DNA, 138 bp, Artificial Sequence
  PgsA7
cacgtatttattgccattccgatcgtttttgtccttatgttcgctttcatgtgggcgggaaaagcggaaacgccgaaggtcaaaacgtattctgacgacgtactctcagcctcatttgtaggcgatattatgatggga

SEQ ID NO: 34 - DNA, 228 bp, Artificial Sequence
  PgsA8
cacgtatttattgccattccgatcgtttttgtccttatgttcgctttcatgtgggcgggaaaagcggaaacgccgaaggtcaaaacgtattctgacgacgtactctcagcctcatttgtaggcgatattatgatgggacgctatgttgaaaaagtaacggagcaaaaaggggcagacagtatttttcaatatgttgaaccgatctttagagcctcggattatgtagca